European Patent Specification EP 3 191 510 B9, published October 4, 2023. Title: Nanobodies suitable for neuron regeneration therapy. Applicant: Institut Pasteur. The sequence listing filed with the application follows.

SEQUENCE LISTING (49 sequences)

SEQ ID NO: 1 - protein, 29 aa, Artificial Sequence
  Synthetic sequence
YTIWMPENPRLGMSCDIFTNSRGKRASKG

SEQ ID NO: 2 - DNA, 87 bp, Artificial Sequence
  Synthetic sequence
tatacgatttggatgccggaaaatccacgtctgggcatgtcgtgcgatatctttaccaacagtcgcggtaaacgcgcgagcaaaggg

SEQ ID NO: 3 - protein, 120 aa, Artificial Sequence
  Synthetic sequence
EVQLQASGGGLAQPGGSLRLSVTVSGSIDVINNMAWYRQAPGNARELVATITSGFSTNYASSVKGRFTISRDNAKKAVYLQMNSLKPEDTADYYSKVHLIRLGAARAYDYWGQGTQVTVS

SEQ ID NO: 4 - DNA, 360 bp, Artificial Sequence
  Synthetic sequence
gaggtgcagctgcaggcgtctgggggaggcttggcgcagcctggggggtccctgagactctccgtaacagtctctggaagtatcgatgttattaataacatggcctggtaccgccaggctccagggaatgcgcgcgagttggtcgccacaattactagtggttttagcacaaactatgcaagctccgtgaagggccgattcaccatctccagagacaacgccaagaaagcggtatatctacagatgaacagcctgaaacctgaggacacggccgattattactctaaggttcacttaatacgtcttggggccgcgcgggcgtatgactactggggccaggggacccaggtcaccgtctcc

SEQ ID NO: 5 - protein, 16 aa, Artificial Sequence
  Synthetic sequence
GGGSAWSHPQFEKAAA

SEQ ID NO: 6 - DNA, 48 bp, Artificial Sequence
  Synthetic sequence
ggtggaggctcagcttggagccacccgcagttcgaaaaagcggccgca

SEQ ID NO: 7 - protein, 42 aa, Artificial Sequence
  Synthetic sequence
RRVNRSEPTQHNLRGTGREVSVTPQSGKIISSWEVHGQQTRL

SEQ ID NO: 8 - DNA, 126 bp, Artificial Sequence
  Synthetic sequence
cgccgggtaaaccgcagtgaaccgacccagcacaatctgcgtgggactggtcgtgaggtgtccgttacgccacagtctggcaaaatcattagctcgtgggaagtacatggccagcaaacccgctta

SEQ ID NO: 9 - protein, 38 aa, Artificial Sequence
  Synthetic sequence
RRVNRSEPTQHNLRGTGREVSVTPQSGKIISSWEVHGQ

SEQ ID NO: 10 - DNA, 114 bp, Artificial Sequence
  Synthetic sequence
cgccgggtaaaccgcagtgaaccgacccagcacaatctgcgtgggactggtcgtgaggtgtccgttacgccacagtctggcaaaatcattagctcgtgggaagtacatggccag

SEQ ID NO: 11 - protein, 209 aa, Artificial Sequence
  Synthetic sequence
MAYTIWMPENPRLGMSCDIFTNSRGKRASKGEVQLQASGGGLAQPGGSLRLSVTVSGSIDVINNMAWYRQAPGNARELVATITSGFSTNYASSVKGRFTISRDNAKKAVYLQMNSLKPEDTADYYSKVHLIRLGAARAYDYWGQGTQVTVSGGGSAWSHPQFEKAAARRVNRSEPTQHNLRGTGREVSVTPQSGKIISSWEVHGQQTRL

SEQ ID NO: 12 - DNA, 633 bp, Artificial Sequence
  Synthetic sequence
atggcctatacgatttggatgccggaaaatccacgtctgggcatgtcgtgcgatatctttaccaacagtcgcggtaaacgcgcgagcaaaggggaggtgcagctgcaggcgtctgggggaggcttggcgcagcctggggggtccctgagactctccgtaacagtctctggaagtatcgatgttattaataacatggcctggtaccgccaggctccagggaatgcgcgcgagttggtcgccacaattactagtggttttagcacaaactatgcaagctccgtgaagggccgattcaccatctccagagacaacgccaagaaagcggtatatctacagatgaacagcctgaaacctgaggacacggccgattattactctaaggttcacttaatacgtcttggggccgcgcgggcgtatgactactggggccaggggacccaggtcaccgtctccggtggaggctcagcttggagccacccgcagttcgaaaaagcggccgcacgccgggtaaaccgcagtgaaccgacccagcacaatctgcgtgggactggtcgtgaggtgtccgttacgccacagtctggcaaaatcattagctcgtgggaagtacatggccagcaaacccgcttatgataa

SEQ ID NO: 13 - protein, 180 aa, Artificial Sequence
  Synthetic sequence
MAEVQLQASGGGLAQPGGSLRLSVTVSGSIDVINNMAWYRQAPGNARELVATITSGFSTNYASSVKGRFTISRDNAKKAVYLQMNSLKPEDTADYYSKVHLIRLGAARAYDYWGQGTQVTVSGGGSAWSHPQFEKAAARRVNRSEPTQHNLRGTGREVSVTPQSGKIISSWEVHGQQTRL

SEQ ID NO: 14 - DNA, 546 bp, Artificial Sequence
  Synthetic sequence
atggccgaggtgcagctgcaggcgtctgggggaggcttggcgcagcctggggggtccctgagactctccgtaacagtctctggaagtatcgatgttattaataacatggcctggtaccgccaggctccagggaatgcgcgcgagttggtcgccacaattactagtggttttagcacaaactatgcaagctccgtgaagggccgattcaccatctccagagacaacgccaagaaagcggtatatctacagatgaacagcctgaaacctgaggacacggccgattattactctaaggttcacttaatacgtcttggggccgcgcgggcgtatgactactggggccaggggacccaggtcaccgtctccggtggaggctcagcttggagccacccgcagttcgaaaaagcggccgcacgccgggtaaaccgcagtgaaccgacccagcacaatctgcgtgggactggtcgtgaggtgtccgttacgccacagtctggcaaaatcattagctcgtgggaagtacatggccagcaaacccgcttatgataa

SEQ ID NO: 15 - protein, 205 aa, Artificial Sequence
  Synthetic sequence
MAYTIWMPENPRLGMSCDIFTNSRGKRASKGEVQLQASGGGLAQPGGSLRLSVTVSGSIDVINNMAWYRQAPGNARELVATITSGFSTNYASSVKGRFTISRDNAKKAVYLQMNSLKPEDTADYYSKVHLIRLGAARAYDYWGQGTQVTVSGGGSAWSHPQFEKAAARRVNRSEPTQHNLRGTGREVSVTPQSGKIISSWEVHGQ

SEQ ID NO: 16 - DNA, 621 bp, Artificial Sequence
  Synthetic sequence
atggcctatacgatttggatgccggaaaatccacgtctgggcatgtcgtgcgatatctttaccaacagtcgcggtaaacgcgcgagcaaaggggaggtgcagctgcaggcgtctgggggaggcttggcgcagcctggggggtccctgagactctccgtaacagtctctggaagtatcgatgttattaataacatggcctggtaccgccaggctccagggaatgcgcgcgagttggtcgccacaattactagtggttttagcacaaactatgcaagctccgtgaagggccgattcaccatctccagagacaacgccaagaaagcggtatatctacagatgaacagcctgaaacctgaggacacggccgattattactctaaggttcacttaatacgtcttggggccgcgcgggcgtatgactactggggccaggggacccaggtcaccgtctccggtggaggctcagcttggagccacccgcagttcgaaaaagcggccgcacgccgggtaaaccgcagtgaaccgacccagcacaatctgcgtgggactggtcgtgaggtgtccgttacgccacagtctggcaaaatcattagctcgtgggaagtacatggccagtgataa

SEQ ID NO: 17 - protein, 31 aa, Artificial Sequence
  Synthetic sequence
RRVNRSEPTQHNLRGTGREVSVTPQSGKIIS

SEQ ID NO: 18 - protein, 31 aa, Artificial Sequence
  Synthetic sequence
RRVNRSEPTQLNLRGTGREVSVTPQSGKIIS

SEQ ID NO: 19 - protein, 13 aa, Artificial Sequence
  Synthetic sequence
SWESHKSGGQTRL

SEQ ID NO: 20 - protein, 44 aa, Artificial Sequence
  Synthetic sequence
RRVNRSEPTQHNLRGTGREVSVTPQSGKIISSWESHKSGGQTRL

SEQ ID NO: 21 - protein, 11 aa, Artificial Sequence
  Synthetic sequence
  misc_feature (3)..(7): Xaa can be any naturally occurring amino acid
SWXXXXXQTRL

SEQ ID NO: 22 - protein, 12 aa, Artificial Sequence
  Synthetic sequence
  misc_feature (3)..(8): Xaa can be any naturally occurring amino acid
SWXXXXXXQTRL

SEQ ID NO: 23 - protein, 13 aa, Artificial Sequence
  Synthetic sequence
  misc_feature (3)..(9): Xaa can be any naturally occurring amino acid
SWXXXXXXXQTRL

SEQ ID NO: 24 - protein, 42 aa, Artificial Sequence
  Synthetic sequence
RRVNRSEPTQHNLRGTGREVSVTPQSGKIISSWEVHGGQTRL

SEQ ID NO: 25 - protein, 42 aa, Artificial Sequence
  Synthetic sequence
RRVNRSEPTQHNLRGTGREVSVTPQSGKIISSWEVATQQTRL

SEQ ID NO: 26 - protein, 42 aa, Artificial Sequence
  Synthetic sequence
RRVNRSEPTQHNLRGTGREVSVTPQSGKIISSWEVYTGQTRL

SEQ ID NO: 27 - protein, 42 aa, Artificial Sequence
  Synthetic sequence
RRVNRSEPTQHNLRGTGREVSVTPQSGKIISSWEVHTGQTRL

SEQ ID NO: 28 - protein, 42 aa, Artificial Sequence
  Synthetic sequence
RRVNRSEPTQHNLRGTGREVSVTPQSGKIISSWEVHTQQTRL

SEQ ID NO: 29 - protein, 42 aa, Artificial Sequence
  Synthetic sequence
RRVNRSEPTQHNLRGTGREVSVTPQSGKIISSWEVAGGQTRL

SEQ ID NO: 30 - protein, 44 aa, Artificial Sequence
  Synthetic sequence
RRVNRSEPTQHNLRGTGREVSVTPQSGKIISSWAEAQHTQQTRL

SEQ ID NO: 31 - protein, 44 aa, Artificial Sequence
  Synthetic sequence
RRVNRSEPTQHNLRGTGREVSVTPQSGKIISSWEVHASGGQTRL

SEQ ID NO: 32 - protein, 30 aa, Artificial Sequence
  Synthetic sequence
KSVRTWNEILPSKGCLRVGGRCHPHVNGGG

SEQ ID NO: 33 - protein, 25 aa, Artificial Sequence
  Synthetic sequence
KSVRTWNEIIPSKGCLRVGGRCHPH

SEQ ID NO: 34 - protein, 29 aa, Artificial Sequence
  Synthetic sequence
YTIWMPENPRPGTPCDIFTNSRGKRASNG

SEQ ID NO: 35 - protein, 24 aa, Artificial Sequence
  Synthetic sequence
GGTATAGTCAATTCTTATTTGAAT

SEQ ID NO: 36 - protein, 24 aa, Artificial Sequence
  Synthetic sequence
CTTGAATCTCAATAGGTGCCCTTA

SEQ ID NO: 37 - protein, 23 aa, Artificial Sequence
  Synthetic sequence
TTAACACTTCATGGCCTGTAAGA

SEQ ID NO: 38 - protein, 24 aa, Artificial Sequence
  Synthetic sequence
TGTGCCATTGCTCCAGTATTCTTG

SEQ ID NO: 39 - protein, 24 aa, Artificial Sequence
  Synthetic sequence
CTGCTTCTTAACCCCAGTAAGCCA

SEQ ID NO: 40 - protein, 24 aa, Artificial Sequence
  Synthetic sequence
CAGCAGTGCCCTGAAGATTAGCAG

SEQ ID NO: 41 - protein, 24 aa, Artificial Sequence
  Synthetic sequence
CCCCAGGCGATGGACAATTATGAT

SEQ ID NO: 42 - protein, 24 aa, Artificial Sequence
  Synthetic sequence
CACTTGGTTTTATTGCACAGAAGC

SEQ ID NO: 43 - protein, 24 aa, Artificial Sequence
  Synthetic sequence
TCCTGCTGTGTCCTGAGGTGCATT

SEQ ID NO: 44 - protein, 24 aa, Artificial Sequence
  Synthetic sequence
GCCCAGATCCAGCATGCAAGGTGC

SEQ ID NO: 45 - protein, 193 aa, Artificial Sequence
  Synthetic sequence
MAYTIWMPENPRLGMSCDIFTNSRGKRASKGEVQLQASGGGLAQPGGSLRLSVTVSGSIDVINNMAWYRQAPGNARELVATITSGFSTNYASSVKGRFTISRDNAKKAVYLQMNSLKPEDTADYYSKVHLIRLGAARAYDYWGQGTQVTVSRRVNRSEPTQHNLRGTGREVSVTPQSGKIISSWEVHGQQTRL

SEQ ID NO: 46 - DNA, 585 bp, Artificial Sequence
  Synthetic sequence
atggcctatacgatttggatgccggaaaatccacgtctgggcatgtcgtgcgatatctttaccaacagtcgcggtaaacgcgcgagcaaaggggaggtgcagctgcaggcgtctgggggaggcttggcgcagcctggggggtccctgagactctccgtaacagtctctggaagtatcgatgttattaataacatggcctggtaccgccaggctccagggaatgcgcgcgagttggtcgccacaattactagtggttttagcacaaactatgcaagctccgtgaagggccgattcaccatctccagagacaacgccaagaaagcggtatatctacagatgaacagcctgaaacctgaggacacggccgattattactctaaggttcacttaatacgtcttggggccgcgcgggcgtatgactactggggccaggggacccaggtcaccgtctcccgccgggtaaaccgcagtgaaccgacccagcacaatctgcgtgggactggtcgtgaggtgtccgttacgccacagtctggcaaaatcattagctcgtgggaagtacatggccagcaaacccgcttatgataa

SEQ ID NO: 47 - protein, 8 aa, Artificial Sequence
  Synthetic sequence
IDVINNMA

SEQ ID NO: 48 - protein, 10 aa, Artificial Sequence
  Synthetic sequence
TITSGFSTNY

SEQ ID NO: 49 - protein, 15 aa, Artificial Sequence
  Synthetic sequence
KVHLIRLGAARAYDY